European Patent Specification EP 3 794 146 B1, published December 10, 2025. Title: CHEMICAL COMPOSITIONS AND METHODS OF USING SAME. Applicant: NanoString Technologies, Inc. Dunaway, Dwayne Hoang, Margaret Gregory, Mark Kim, Dae Manrao, Elizabeth A Beechem, Joseph M Walsh, Matthew Khafizov, Rustem Korukonda, Sanghamithra Deng, Yi Meredith, Gavin McElwain, Mark Skene, Peter Burke, Cassandra. The sequence listing filed with the application follows.

SEQUENCE LISTING (114 sequences)

SEQ ID NO: 1 - DNA, 38 bp, Homo sapiens
accgtgacatgagaagaacaggtcgacataggtcatac

SEQ ID NO: 2 - DNA, 10 bp, Artificial Sequence
  Example Consensus
aacaccacct

SEQ ID NO: 3 - DNA, 24 bp, Homo sapiens
gtctagctacagtgaaatctcgat

SEQ ID NO: 4 - DNA, 23 bp, Homo sapiens
tcaaagtgctgggctccggtgcg

SEQ ID NO: 5 - DNA, 27 bp, Homo sapiens
tagttggagctggtggcgtaggcaaga

SEQ ID NO: 6 - DNA, 23 bp, Homo sapiens
gaatgatgcacatcatggtggct

SEQ ID NO: 7 - DNA, 23 bp, Homo sapiens
gcagctcatcacgcagctcatgc

SEQ ID NO: 8 - DNA, 23 bp, Homo sapiens
atacagctggacaagaagagtac

SEQ ID NO: 9 - DNA, 25 bp, Homo sapiens
tggctcgagatatcatgagtgattc

SEQ ID NO: 10 - DNA, 23 bp, Homo sapiens
tcatcataggtcgtcatgcttat

SEQ ID NO: 11 - DNA, 23 bp, Homo sapiens
atggagtatgtgtctgtggagac

SEQ ID NO: 12 - DNA, 23 bp, Homo sapiens
gtgcaactctccgtacatcgtgg

SEQ ID NO: 13 - DNA, 23 bp, Homo sapiens
cagccgcgtgctgcacaccaacg

SEQ ID NO: 14 - RNA, 30 nt, Homo sapiens
gcuucagcaccacuccacuccacauucuca

SEQ ID NO: 15 - RNA, 30 nt, Homo sapiens
uguccucauguauuggucucucauggcacu

SEQ ID NO: 16 - RNA, 30 nt, Homo sapiens
cuuucgccaaaguggaggagaccaucgccg

SEQ ID NO: 17 - RNA, 30 nt, Homo sapiens
gaaggugauguuugggucaggugccuuagu

SEQ ID NO: 18 - DNA, 50 bp, Homo sapiens
caaactggtggtggttggagcaggtggtgttgggaaaagcgcactgacaa

SEQ ID NO: 19 - DNA, 12 bp, Artificial Sequence
  12-mer attachment position
aggacagatgac

SEQ ID NO: 20 - DNA, 12 bp, Artificial Sequence
  12-mer attachment position
gtatcggatgac

SEQ ID NO: 21 - DNA, 12 bp, Artificial Sequence
  12-mer attachment position
aggagtgatgac

SEQ ID NO: 22 - DNA, 12 bp, Artificial Sequence
  12-mer attachment position
aggggtgaggag

SEQ ID NO: 23 - DNA, 12 bp, Artificial Sequence
  12-mer attachment position
agaggggatgac

SEQ ID NO: 24 - DNA, 12 bp, Artificial Sequence
  12-mer attachment position
agtggggaggag

SEQ ID NO: 25 - DNA, 12 bp, Artificial Sequence
  12-mer attachment position
agccgagatgac

SEQ ID NO: 26 - DNA, 12 bp, Artificial Sequence
  12-mer attachment position
agggtggatgac

SEQ ID NO: 27 - DNA, 12 bp, Artificial Sequence
  12-mer attachment position
tggatggaaaag

SEQ ID NO: 28 - DNA, 12 bp, Artificial Sequence
  12-mer attachment position
gaaggagaaaag

SEQ ID NO: 29 - DNA, 12 bp, Artificial Sequence
  12-mer attachment position
ggggatgaaaag

SEQ ID NO: 30 - DNA, 12 bp, Artificial Sequence
  12-mer attachment position
gtgagggaaaag

SEQ ID NO: 31 - DNA, 12 bp, Artificial Sequence
  12-mer attachment position
agccgagaaaag

SEQ ID NO: 32 - DNA, 12 bp, Artificial Sequence
  12-mer attachment position
cgagaggaaaag

SEQ ID NO: 33 - DNA, 12 bp, Artificial Sequence
  12-mer attachment position
gagggcgaaaag

SEQ ID NO: 34 - DNA, 12 bp, Artificial Sequence
  12-mer attachment position
agcgtggaaaag

SEQ ID NO: 35 - DNA, 12 bp, Artificial Sequence
  12-mer attachment position
tgagaagggtag

SEQ ID NO: 36 - DNA, 12 bp, Artificial Sequence
  12-mer attachment position
gttgttattgtg

SEQ ID NO: 37 - DNA, 12 bp, Artificial Sequence
  12-mer attachment position
tttgggtttagg

SEQ ID NO: 38 - DNA, 12 bp, Artificial Sequence
  12-mer attachment position
gttagtgggaaa

SEQ ID NO: 39 - DNA, 12 bp, Artificial Sequence
  12-mer attachment position
atgggaaaaagt

SEQ ID NO: 40 - DNA, 12 bp, Artificial Sequence
  12-mer attachment position
gagttggatgag

SEQ ID NO: 41 - DNA, 12 bp, Artificial Sequence
  12-mer attachment position
atgttgtgggta

SEQ ID NO: 42 - DNA, 12 bp, Artificial Sequence
  12-mer attachment position
gagggttttaag

SEQ ID NO: 43 - DNA, 14 bp, Artificial Sequence
  14-mer attachment position
atcttttccccact

SEQ ID NO: 44 - DNA, 14 bp, Artificial Sequence
  14-mer attachment position
ccccactatttctt

SEQ ID NO: 45 - DNA, 14 bp, Artificial Sequence
  14-mer attachment position
ctacccacaacata

SEQ ID NO: 46 - DNA, 14 bp, Artificial Sequence
  14-mer attachment position
ccatataaacccca

SEQ ID NO: 47 - DNA, 14 bp, Artificial Sequence
  14-mer attachment position
aaactccaatctcc

SEQ ID NO: 48 - DNA, 14 bp, Artificial Sequence
  14-mer attachment position
ctattctcaaccta

SEQ ID NO: 49 - DNA, 14 bp, Artificial Sequence
  14-mer attachment position
ccccctcttttaaa

SEQ ID NO: 50 - DNA, 14 bp, Artificial Sequence
  14-mer attachment position
ccaatcttacctca

SEQ ID NO: 51 - DNA, 14 bp, Artificial Sequence
  14-mer attachment position
ccctcacataactt

SEQ ID NO: 52 - DNA, 14 bp, Artificial Sequence
  14-mer attachment position
ctcctctactttcc

SEQ ID NO: 53 - DNA, 14 bp, Artificial Sequence
  14-mer attachment position
ccctaaacccaaaa

SEQ ID NO: 54 - DNA, 14 bp, Artificial Sequence
  14-mer attachment position
cactttttcccatc

SEQ ID NO: 55 - DNA, 14 bp, Artificial Sequence
  14-mer attachment position
catctgattcctcc

SEQ ID NO: 56 - DNA, 14 bp, Artificial Sequence
  14-mer attachment position
ctaaaccccctact

SEQ ID NO: 57 - DNA, 14 bp, Artificial Sequence
  14-mer attachment position
cctttacaaacaca

SEQ ID NO: 58 - DNA, 14 bp, Artificial Sequence
  14-mer attachment position
ataccaccctcttt

SEQ ID NO: 59 - DNA, 14 bp, Artificial Sequence
  14-mer attachment position
tattcttctacccc

SEQ ID NO: 60 - DNA, 14 bp, Artificial Sequence
  14-mer attachment position
tctacccttctcat

SEQ ID NO: 61 - DNA, 14 bp, Artificial Sequence
  14-mer attachment position
ccacaataacaacc

SEQ ID NO: 62 - DNA, 14 bp, Artificial Sequence
  14-mer attachment position
accttaacattccc

SEQ ID NO: 63 - DNA, 14 bp, Artificial Sequence
  14-mer attachment position
atttcccactaacc

SEQ ID NO: 64 - DNA, 14 bp, Artificial Sequence
  14-mer attachment position
acttaaaaccctcc

SEQ ID NO: 65 - DNA, 14 bp, Artificial Sequence
  14-mer attachment position
tacctattcctcca

SEQ ID NO: 66 - DNA, 14 bp, Artificial Sequence
  14-mer attachment position
cccctttctctaag

SEQ ID NO: 67 - DNA, 14 bp, Artificial Sequence
  14-mer attachment position
gatgatggtaggtg

SEQ ID NO: 68 - DNA, 14 bp, Artificial Sequence
  14-mer attachment position
atgagaagggtaga

SEQ ID NO: 69 - DNA, 14 bp, Artificial Sequence
  14-mer attachment position
gttttgttggtgag

SEQ ID NO: 70 - DNA, 14 bp, Artificial Sequence
  14-mer attachment position
ttagtgtgttggag

SEQ ID NO: 71 - DNA, 14 bp, Artificial Sequence
  14-mer attachment position
atgtaggagagaga

SEQ ID NO: 72 - DNA, 14 bp, Artificial Sequence
  14-mer attachment position
gggaatgttaaggt

SEQ ID NO: 73 - DNA, 14 bp, Artificial Sequence
  14-mer attachment position
ggttagtgggaaat

SEQ ID NO: 74 - DNA, 14 bp, Artificial Sequence
  14-mer attachment position
ggagggttttaagt

SEQ ID NO: 75 - DNA, 14 bp, Artificial Sequence
  14-mer attachment position
gtagtgtggatgtt

SEQ ID NO: 76 - DNA, 14 bp, Artificial Sequence
  14-mer attachment position
cttagagaaagggg

SEQ ID NO: 77 - DNA, 14 bp, Artificial Sequence
  14-mer attachment position
ggaagaggatgaaa

SEQ ID NO: 78 - DNA, 14 bp, Artificial Sequence
  14-mer attachment position
aagttatgtgaggg

SEQ ID NO: 79 - DNA, 14 bp, Artificial Sequence
  14-mer attachment position
ggaaagtagaggag

SEQ ID NO: 80 - DNA, 14 bp, Artificial Sequence
  14-mer attachment position
ttttgggtttaggg

SEQ ID NO: 81 - DNA, 14 bp, Artificial Sequence
  14-mer attachment position
agatgtatgggtga

SEQ ID NO: 82 - DNA, 14 bp, Artificial Sequence
  14-mer attachment position
gatgggaaaaagtg

SEQ ID NO: 83 - DNA, 14 bp, Artificial Sequence
  14-mer attachment position
ggaggaatcagatg

SEQ ID NO: 84 - DNA, 14 bp, Artificial Sequence
  14-mer attachment position
agagggattgatga

SEQ ID NO: 85 - DNA, 14 bp, Artificial Sequence
  14-mer attachment position
tgtgtttgtaaagg

SEQ ID NO: 86 - DNA, 14 bp, Artificial Sequence
  14-mer attachment position
aaggagtgatagga

SEQ ID NO: 87 - DNA, 14 bp, Artificial Sequence
  14-mer attachment position
tggtgatttagagg

SEQ ID NO: 88 - DNA, 14 bp, Artificial Sequence
  14-mer attachment position
ggggtagaagaata

SEQ ID NO: 89 - DNA, 14 bp, Artificial Sequence
  14-mer attachment position
aagaaatagtgggg

SEQ ID NO: 90 - DNA, 14 bp, Artificial Sequence
  14-mer attachment position
tatgttgtgggtag

SEQ ID NO: 91 - DNA, 14 bp, Artificial Sequence
  14-mer attachment position
gttaaagggaggtt

SEQ ID NO: 92 - DNA, 14 bp, Artificial Sequence
  14-mer attachment position
tggggtttatatgg

SEQ ID NO: 93 - DNA, 14 bp, Artificial Sequence
  14-mer attachment position
agggaatatggaga

SEQ ID NO: 94 - DNA, 14 bp, Artificial Sequence
  14-mer attachment position
taggttgagaatag

SEQ ID NO: 95 - DNA, 14 bp, Artificial Sequence
  14-mer attachment position
tttaaaagaggggg

SEQ ID NO: 96 - DNA, 14 bp, Artificial Sequence
  14-mer attachment position
tgaggtaagattgg

SEQ ID NO: 97 - DNA, 10 bp, Artificial Sequence
  Target binding domain
agcttcttat

SEQ ID NO: 98 - DNA, 50 bp, Artificial Sequence
  Target nucleic acid
gagactagcagaataggaggataagaagctcgaagagtgaggacaaatgg

SEQ ID NO: 99 - DNA, 10 bp, Artificial Sequence
  Target binding domain
ttcactgtag

SEQ ID NO: 100 - DNA, 35 bp, Artificial Sequence
  exemplary lawn oligonucleotide
  misc_feature (1)..(1): Modified with a 5' amine with a 6 carbon linker
tggtgaggttgttggtagtagtgagtttgtagggt

SEQ ID NO: 101 - DNA, 25 bp, Artificial Sequence
  exemplary lawn oligonucleotide
  misc_feature (1)..(1): Modified with a 5' amine with a 6 carbon linker
tggtgaggttgttggtagtagtgag

SEQ ID NO: 102 - DNA, 35 bp, Artificial Sequence
  exemplary lawn oligonucleotide
  misc_feature (1)..(1): Modified with a 5' amine with a 6 carbon linker
ttttttttttttttttttttttttttttttttttt

SEQ ID NO: 103 - DNA, 36 bp, Artificial Sequence
  exemplary lawn oligonucleotide
  misc_feature (1)..(1): Modified with a 5' amine with a 6 carbon linker
catctcaaacaccttctacaatatgacctaacacac

SEQ ID NO: 104 - DNA, 36 bp, Artificial Sequence
  exemplary lawn oligonucleotide
  misc_feature (1)..(1): Modified with a 5' amine with a 6 carbon linker
gtgatggttataagaggtgttgatatatttatagta

SEQ ID NO: 105 - DNA, 36 bp, Artificial Sequence
  exemplary lawn oligonucleotide
  misc_feature (1)..(1): Modified with a 5' amine with a 6 carbon linker
tattgatattgagaaagcgtttgatgatgtattgat

SEQ ID NO: 106 - DNA, 36 bp, Artificial Sequence
  exemplary lawn oligonucleotide
  misc_feature (1)..(1): Modified with a 5' amine with a 6 carbon linker
tagttatgtagtagtttgcgaaagagttatagttat

SEQ ID NO: 107 - DNA, 36 bp, Artificial Sequence
  exemplary lawn oligonucleotide
  misc_feature (1)..(1): Modified with a 5' amine with a 6 carbon linker
actaccctactctacccttctaagatatacatatac

SEQ ID NO: 108 - DNA, 35 bp, Artificial Sequence; identical to SEQ ID NO: 100
  exemplary lawn oligonucleotide
  misc_feature (1)..(1): Modified with a 5' amine with a 6 carbon linker
  misc_feature (3)..(3): Comprises isoguanine base
  misc_feature (7)..(7): Comprises isoguanine base
  misc_feature (11)..(11): Comprises isoguanine base
  misc_feature (15)..(15): Comprises isoguanine base
  misc_feature (18)..(18): Comprises isoguanine base
  misc_feature (21)..(21): Comprises isoguanine base
  misc_feature (25)..(25): Comprises isoguanine base
  misc_feature (29)..(29): Comprises isoguanine base
  misc_feature (33)..(33): Comprises isoguanine base

SEQ ID NO: 109 - DNA, 25 bp, Artificial Sequence
  OA-sequence
cgaaagccatgacctccgatcactc

SEQ ID NO: 110 - DNA, 60 bp, Artificial Sequence
  adapter oligonucleotide
  misc_feature (28)..(28): Comprises 5-methyl-isocytosine base
  misc_feature (32)..(32): Comprises 5-methyl-isocytosine base
  misc_feature (36)..(36): Comprises 5-methyl-isocytosine base
  misc_feature (40)..(40): Comprises 5-methyl-isocytosine base
  misc_feature (43)..(43): Comprises 5-methyl-isocytosine base
  misc_feature (46)..(46): Comprises 5-methyl-isocytosine base
  misc_feature (50)..(50): Comprises 5-methyl-isocytosine base
  misc_feature (54)..(54): Comprises 5-methyl-isocytosine base
  misc_feature (58)..(58): Comprises 5-methyl-isocytosine base
gagtgatcggaggtcatggctttcgaccctacaaactcactactaccaacaacctcacca

SEQ ID NO: 111 - DNA, 63 bp, Artificial Sequence
  capture probe
ccggtcaaccgttttgtagaacaactcccgtcccctcactcactagcctccagtaccgaaagc

SEQ ID NO: 112 - DNA, 15 bp, Artificial Sequence
  Single stranded purification sequence
aacatcacacagacc

SEQ ID NO: 113 - DNA, 15 bp, Artificial Sequence
  Single stranded purification sequence
gtctatcatcacagc

SEQ ID NO: 114 - DNA, 34 bp, Artificial Sequence
  lawn oligonucleotide
  misc_feature (1)..(34): L-DNA
tttttttttttttttttttttttttttttttttt